European Patent Specification EP 4 063 521 B1, published February 21, 2024. Title: Method. Applicant: Oxford Nanopore Technologies plc. The sequence listing filed with the application follows.

SEQUENCE LISTING (83 sequences)

SEQ ID NO: 1 - DNA, 558 bp, Artificial Sequence
  MS-B1
atgggtctggataatgaactgagcctggtggacggtcaagatcgtaccctgacggtgcaacaatgggatacctttctgaatggcgtttttccgctggatcgtaatcgcctgacccgtgaatggtttcattccggtcgcgcaaaatatatcgtcgcaggcccgggtgctgacgaattcgaaggcacgctggaactgggttatcagattggctttccgtggtcactgggcgttggtatcaacttctcgtacaccacgccgaatattctgatcaacaatggtaacattaccgcaccgccgtttggcctgaacagcgtgattacgccgaacctgtttccgggtgttagcatctctgcccgtctgggcaatggtccgggcattcaagaagtggcaacctttagtgtgcgcgtttccggcgctaaaggcggtgtcgcggtgtctaacgcccacggtaccgttacgggcgcggccggcggtgtcctgctgcgtccgttcgcgcgcctgattgcctctaccggcgacagcgttacgacctatggcgaaccgtggaatatgaactaa

SEQ ID NO: 2 - protein, 184 aa, Artificial Sequence
  MS-B1
GLDNELSLVDGQDRTLTVQQWDTFLNGVFPLDRNRLTREWFHSGRAKYIVAGPGADEFEGTLELGYQIGFPWSLGVGINFSYTTPNILINNGNITAPPFGLNSVITPNLFPGVSISARLGNGPGIQEVATFSVRVSGAKGGVAVSNAHGTVTGAAGGVLLRPFARLIASTGDSVTTYGEPWNMN

SEQ ID NO: 3 - DNA, 885 bp, Artificial Sequence
  alpha-HL-NN
atggcagattctgatattaatattaaaaccggtactacagatattggaagcaatactacagtaaaaacaggtgatttagtcacttatgataaagaaaatggcatgcacaaaaaagtattttatagttttatcgatgataaaaatcacaataaaaaactgctagttattagaacaaaaggtaccattgctggtcaatatagagtttatagcgaagaaggtgctaacaaaagtggtttagcctggccttcagcctttaaggtacagttgcaactacctgataatgaagtagctcaaatatctgattactatccaagaaattcgattgatacaaaaaactatatgagtactttaacttatggattcaacggtaatgttactggtgatgatacaggaaaaattggcggccttattggtgcaaatgtttcgattggtcatacactgaactatgttcaacctgatttcaaaacaattttagagagcccaactgataaaaaagtaggctggaaagtgatatttaacaatatggtgaatcaaaattggggaccatacgatcgagattcttggaacccggtatatggcaatcaacttttcatgaaaactagaaatggttctatgaaagcagcagataacttccttgatcctaacaaagcaagttctctattatcttcagggttttcaccagacttcgctacagttattactatggatagaaaagcatccaaacaacaaacaaatatagatgtaatatacgaacgagttcgtgatgattaccaattgcattggacttcaacaaattggaaaggtaccaatactaaagataaatggacagatcgttcttcagaaagatataaaatcgattgggaaaaagaagaaatgacaaattaa

SEQ ID NO: 4 - protein, 293 aa, Artificial Sequence
  alpha-HL-NN
ADSDINIKTGTTDIGSNTTVKTGDLVTYDKENGMHKKVFYSFIDDKNHNKKLLVIRTKGTIAGQYRVYSEEGANKSGLAWPSAFKVQLQLPDNEVAQISDYYPRNSIDTKNYMSTLTYGFNGNVTGDDTGKIGGLIGANVSIGHTLNYVQPDFKTILESPTDKKVGWKVIFNNMVNQNWGPYDRDSWNPVYGNQLFMKTRNGSMKAADNFLDPNKASSLLSSGFSPDFATVITMDRKASKQQTNIDVIYERVRDDYQLHWTSTNWKGTNTKDKWTDRSSERYKIDWEKEEMTN

SEQ ID NO: 5 - protein, 184 aa, Artificial Sequence
  MspB
GLDNELSLVDGQDRTLTVQQWDTFLNGVFPLDRNRLTREWFHSGRAKYIVAGPGADEFEGTLELGYQIGFPWSLGVGINFSYTTPNILIDDGDITAPPFGLNSVITPNLFPGVSISADLGNGPGIQEVATFSVDVSGPAGGVAVSNAHGTVTGAAGGVLLRPFARLIASTGDSVTTYGEPWNMN

SEQ ID NO: 6 - protein, 184 aa, Artificial Sequence
  MspC
GLDNELSLVDGQDRTLTVQQWDTFLNGVFPLDRNRLTREWFHSGRAKYIVAGPGADEFEGTLELGYQIGFPWSLGVGINFSYTTPNILIDDGDITGPPFGLESVITPNLFPGVSISADLGNGPGIQEVATFSVDVSGPAGGVAVSNAHGTVTGAAGGVLLRPFARLIASTGDSVTTYGEPWNMN

SEQ ID NO: 7 - protein, 183 aa, Artificial Sequence
  MspD
VDNQLSVVDGQGRTLTVQQAETFLNGVFPLDRNRLTREWFHSGRATYHVAGPGADEFEGTLELGYQVGFPWSLGVGINFSYTTPNILIDGGDITQPPFGLDTIITPNLFPGVSISADLGNGPGIQEVATFSVDVKGAKGAVAVSNAHGTVTGAAGGVLLRPFARLIASTGDSVTTYGEPWNMN

SEQ ID NO: 8 - DNA, 1830 bp, Artificial Sequence
  Phi29 DNA polymerase
atgaaacacatgccgcgtaaaatgtatagctgcgcgtttgaaaccacgaccaaagtggaagattgtcgcgtttgggcctatggctacatgaacatcgaagatcattctgaatacaaaatcggtaacagtctggatgaatttatggcatgggtgctgaaagttcaggcggatctgtacttccacaacctgaaatttgatggcgcattcattatcaactggctggaacgtaatggctttaaatggagcgcggatggtctgccgaacacgtataataccattatctctcgtatgggccagtggtatatgattgatatctgcctgggctacaaaggtaaacgcaaaattcataccgtgatctatgatagcctgaaaaaactgccgtttccggtgaagaaaattgcgaaagatttcaaactgacggttctgaaaggcgatattgattatcacaaagaacgtccggttggttacaaaatcaccccggaagaatacgcatacatcaaaaacgatatccagatcatcgcagaagcgctgctgattcagtttaaacagggcctggatcgcatgaccgcgggcagtgatagcctgaaaggtttcaaagatatcatcacgaccaaaaaattcaaaaaagtgttcccgacgctgagcctgggtctggataaagaagttcgttatgcctaccgcggcggttttacctggctgaacgatcgtttcaaagaaaaagaaattggcgagggtatggtgtttgatgttaatagtctgtatccggcacagatgtacagccgcctgctgccgtatggcgaaccgatcgtgttcgagggtaaatatgtttgggatgaagattacccgctgcatattcagcacatccgttgtgaatttgaactgaaagaaggctatattccgaccattcagatcaaacgtagtcgcttctataagggtaacgaatacctgaaaagctctggcggtgaaatcgcggatctgtggctgagtaacgtggatctggaactgatgaaagaacactacgatctgtacaacgttgaatacatcagcggcctgaaatttaaagccacgaccggtctgttcaaagatttcatcgataaatggacctacatcaaaacgacctctgaaggcgcgattaaacagctggccaaactgatgctgaacagcctgtatggcaaattcgcctctaatccggatgtgaccggtaaagttccgtacctgaaagaaaatggcgcactgggttttcgcctgggcgaagaagaaacgaaagatccggtgtataccccgatgggtgttttcattacggcctgggcacgttacacgaccatcaccgcggcccaggcatgctatgatcgcattatctactgtgataccgattctattcatctgacgggcaccgaaatcccggatgtgattaaagatatcgttgatccgaaaaaactgggttattgggcccacgaaagtacgtttaaacgtgcaaaatacctgcgccagaaaacctacatccaggatatctacatgaaagaagtggatggcaaactggttgaaggttctccggatgattacaccgatatcaaattcagtgtgaaatgcgccggcatgacggataaaatcaaaaaagaagtgaccttcgaaaacttcaaagttggtttcagccgcaaaatgaaaccgaaaccggtgcaggttccgggcggtgtggttctggtggatgatacgtttaccattaaatctggcggtagtgcgtggagccatccgcagttcgaaaaaggcggtggctctggtggcggttctggcggtagtgcctggagccacccgcagtttgaaaaataataa

SEQ ID NO: 9 - protein, 608 aa, Artificial Sequence
  Phi29 DNA polymerase
MKHMPRKMYSCAFETTTKVEDCRVWAYGYMNIEDHSEYKIGNSLDEFMAWVLKVQADLYFHNLKFDGAFIINWLERNGFKWSADGLPNTYNTIISRMGQWYMIDICLGYKGKRKIHTVIYDSLKKLPFPVKKIAKDFKLTVLKGDIDYHKERPVGYKITPEEYAYIKNDIQIIAEALLIQFKQGLDRMTAGSDSLKGFKDIITTKKFKKVFPTLSLGLDKEVRYAYRGGFTWLNDRFKEKEIGEGMVFDVNSLYPAQMYSRLLPYGEPIVFEGKYVWDEDYPLHIQHIRCEFELKEGYIPTIQIKRSRFYKGNEYLKSSGGEIADLWLSNVDLELMKEHYDLYNVEYISGLKFKATTGLFKDFIDKWTYIKTTSEGAIKQLAKLMLNSLYGKFASNPDVTGKVPYLKENGALGFRLGEEETKDPVYTPMGVFITAWARYTTITAAQACYDRIIYCDTDSIHLTGTEIPDVIKDIVDPKKLGYWAHESTFKRAKYLRQKTYIQDIYMKEVDGKLVEGSPDDYTDIKFSVKCAGMTDKIKKEVTFENFKVGFSRKMKPKPVQVPGGVVLVDDTFTIKSGGSAWSHPQFEKGGGSGGGSGGSAWSHPQFEK

SEQ ID NO: 10 - DNA, 1390 bp, Artificial Sequence
  WT EcoExo I
atgatgaacgatggcaaacagcagagcaccttcctgtttcatgattatgaaaccttcggtacccatccggccctggatcgtccggcgcagtttgcggccattcgcaccgatagcgaattcaatgtgattggcgaaccggaagtgttttattgcaaaccggccgatgattatctgccgcagccgggtgcggtgctgattaccggtattaccccgcaggaagcgcgcgcgaaaggtgaaaacgaagcggcgtttgccgcgcgcattcatagcctgtttaccgtgccgaaaacctgcattctgggctataacaatgtgcgcttcgatgatgaagttacccgtaatatcttttatcgtaacttttatgatccgtatgcgtggagctggcagcatgataacagccgttgggatctgctggatgtgatgcgcgcgtgctatgcgctgcgcccggaaggcattaattggccggaaaacgatgatggcctgccgagctttcgtctggaacatctgaccaaagccaacggcattgaacatagcaatgcccatgatgcgatggccgatgtttatgcgaccattgcgatggcgaaactggttaaaacccgtcagccgcgcctgtttgattatctgtttacccaccgtaacaaacacaaactgatggcgctgattgatgttccgcagatgaaaccgctggtgcatgtgagcggcatgtttggcgcctggcgcggcaacaccagctgggtggccccgctggcctggcacccggaaaatcgtaacgccgtgattatggttgatctggccggtgatattagcccgctgctggaactggatagcgataccctgcgtgaacgcctgtataccgccaaaaccgatctgggcgataatgccgccgtgccggtgaaactggttcacattaacaaatgcccggtgctggcccaggcgaacaccctgcgcccggaagatgcggatcgtctgggtattaatcgccagcattgtctggataatctgaaaatcctgcgtgaaaacccgcaggtgcgtgaaaaagtggtggcgatcttcgcggaagcggaaccgttcaccccgagcgataacgtggatgcgcagctgtataacggcttctttagcgatgccgatcgcgcggcgatgaaaatcgttctggaaaccgaaccgcgcaatctgccggcgctggatattacctttgttgataaacgtattgaaaaactgctgtttaattatcgtgcgcgcaattttccgggtaccctggattatgccgaacagcagcgttggctggaacatcgtcgtcaggttttcaccccggaatttctgcagggttatgcggatgaactgcagatgctggttcagcagtatgccgatgataaagaaaaagtggcgctgc

SEQ ID NO: 11 - protein, 485 aa, Artificial Sequence
  WT EcoExo I
MMNDGKQQSTFLFHDYETFGTHPALDRPAQFAAIRTDSEFNVIGEPEVFYCKPADDYLPQPGAVLITGITPQEARAKGENEAAFAARIHSLFTVPKTCILGYNNVRFDDEVTRNIFYRNFYDPYAWSWQHDNSRWDLLDVMRACYALRPEGINWPENDDGLPSFRLEHLTKANGIEHSNAHDAMADVYATIAMAKLVKTRQPRLFDYLFTHRNKHKLMALIDVPQMKPLVHVSGMFGAWRGNTSWVAPLAWHPENRNAVIMVDLAGDISPLLELDSDTLRERLYTAKTDLGDNAAVPVKLVHINKCPVLAQANTLRPEDADRLGINRQHCLDNLKILRENPQVREKVVAIFAEAEPFTPSDNVDAQLYNGFFSDADRAAMKIVLETEPRNLPALDITFVDKRIEKLLFNYRARNFPGTLDYAEQQRWLEHRRQVFTPEFLQGYADELQMLVQQYADDKEKVALLKALWQYAEEIVSGSGHHHHHH

SEQ ID NO: 12 - DNA, 804 bp, Artificial Sequence
  exonuclease III enzyme from E. coli
atgaaatttgtctcttttaatatcaacggcctgcgcgccagacctcaccagcttgaagccatcgtcgaaaagcaccaaccggatgtgattggcctgcaggagacaaaagttcatgacgatatgtttccgctcgaagaggtggcgaagctcggctacaacgtgttttatcacgggcagaaaggccattatggcgtggcgctgctgaccaaagagacgccgattgccgtgcgtcgcggctttcccggtgacgacgaagaggcgcagcggcggattattatggcggaaatcccctcactgctgggtaatgtcaccgtgatcaacggttacttcccgcagggtgaaagccgcgaccatccgataaaattcccggcaaaagcgcagttttatcagaatctgcaaaactacctggaaaccgaactcaaacgtgataatccggtactgattatgggcgatatgaatatcagccctacagatctggatatcggcattggcgaagaaaaccgtaagcgctggctgcgtaccggtaaatgctctttcctgccggaagagcgcgaatggatggacaggctgatgagctgggggttggtcgataccttccgccatgcgaatccgcaaacagcagatcgtttctcatggtttgattaccgctcaaaaggttttgacgataaccgtggtctgcgcatcgacctgctgctcgccagccaaccgctggcagaatgttgcgtagaaaccggcatcgactatgaaatccgcagcatggaaaaaccgtccgatcacgcccccgtctgggcgaccttccgccgc

SEQ ID NO: 13 - protein, 268 aa, Artificial Sequence
  exonuclease III enzyme from E. coli
MKFVSFNINGLRARPHQLEAIVEKHQPDVIGLQETKVHDDMFPLEEVAKLGYNVFYHGQKGHYGVALLTKETPIAVRRGFPGDDEEAQRRIIMAEIPSLLGNVTVINGYFPQGESRDHPIKFPAKAQFYQNLQNYLETELKRDNPVLIMGDMNISPTDLDIGIGEENRKRWLRTGKCSFLPEEREWMDRLMSWGLVDTFRHANPQTADRFSWFDYRSKGFDDNRGLRIDLLLASQPLAECCVETGIDYEIRSMEKPSDHAPVWATFRR

SEQ ID NO: 14 - DNA, 1275 bp, Artificial Sequence
  TthRecJ-cd
atgtttcgtcgtaaagaagatctggatccgccgctggcactgctgccgctgaaaggcctgcgcgaagccgccgcactgctggaagaagcgctgcgtcaaggtaaacgcattcgtgttcacggcgactatgatgcggatggcctgaccggcaccgcgatcctggttcgtggtctggccgccctgggtgcggatgttcatccgtttatcccgcaccgcctggaagaaggctatggtgtcctgatggaacgcgtcccggaacatctggaagcctcggacctgtttctgaccgttgactgcggcattaccaaccatgcggaactgcgcgaactgctggaaaatggcgtggaagtcattgttaccgatcatcatacgccgggcaaaacgccgccgccgggtctggtcgtgcatccggcgctgacgccggatctgaaagaaaaaccgaccggcgcaggcgtggcgtttctgctgctgtgggcactgcatgaacgcctgggcctgccgccgccgctggaatacgcggacctggcagccgttggcaccattgccgacgttgccccgctgtggggttggaatcgtgcactggtgaaagaaggtctggcacgcatcccggcttcatcttgggtgggcctgcgtctgctggctgaagccgtgggctataccggcaaagcggtcgaagtcgctttccgcatcgcgccgcgcatcaatgcggcttcccgcctgggcgaagcggaaaaagccctgcgcctgctgctgacggatgatgcggcagaagctcaggcgctggtcggcgaactgcaccgtctgaacgcccgtcgtcagaccctggaagaagcgatgctgcgcaaactgctgccgcaggccgacccggaagcgaaagccatcgttctgctggacccggaaggccatccgggtgttatgggtattgtggcctctcgcatcctggaagcgaccctgcgcccggtctttctggtggcccagggcaaaggcaccgtgcgttcgctggctccgatttccgccgtcgaagcactgcgcagcgcggaagatctgctgctgcgttatggtggtcataaagaagcggcgggtttcgcaatggatgaagcgctgtttccggcgttcaaagcacgcgttgaagcgtatgccgcacgtttcccggatccggttcgtgaagtggcactgctggatctgctgccggaaccgggcctgctgccgcaggtgttccgtgaactggcactgctggaaccgtatggtgaaggtaacccggaaccgctgttcctg

SEQ ID NO: 15 - protein, 425 aa, Artificial Sequence
  TthRecJ-cd
MFRRKEDLDPPLALLPLKGLREAAALLEEALRQGKRIRVHGDYDADGLTGTAILVRGLAALGADVHPFIPHRLEEGYGVLMERVPEHLEASDLFLTVDCGITNHAELRELLENGVEVIVTDHHTPGKTPPPGLVVHPALTPDLKEKPTGAGVAFLLLWALHERLGLPPPLEYADLAAVGTIADVAPLWGWNRALVKEGLARIPASSWVGLRLLAEAVGYTGKAVEVAFRIAPRINAASRLGEAEKALRLLLTDDAAEAQALVGELHRLNARRQTLEEAMLRKLLPQADPEAKAIVLLDPEGHPGVMGIVASRILEATLRPVFLVAQGKGTVRSLAPISAVEALRSAEDLLLRYGGHKEAAGFAMDEALFPAFKARVEAYAARFPDPVREVALLDLLPEPGLLPQVFRELALLEPYGEGNPEPLFL

SEQ ID NO: 16 - DNA, 738 bp, Artificial Sequence
  bacteriophage lambda exo (redX)
tccggaagcggctctggtagtggttctggcatgacaccggacattatcctgcagcgtaccgggatcgatgtgagagctgtcgaacagggggatgatgcgtggcacaaattacggctcggcgtcatcaccgcttcagaagttcacaacgtgatagcaaaaccccgctccggaaagaagtggcctgacatgaaaatgtcctacttccacaccctgcttgctgaggtttgcaccggtgtggctccggaagttaacgctaaagcactggcctggggaaaacagtacgagaacgacgccagaaccctgtttgaattcacttccggcgtgaatgttactgaatccccgatcatctatcgcgacgaaagtatgcgtaccgcctgctctcccgatggtttatgcagtgacggcaacggccttgaactgaaatgcccgtttacctcccgggatttcatgaagttccggctcggtggtttcgaggccataaagtcagcttacatggcccaggtgcagtacagcatgtgggtgacgcgaaaaaatgcctggtactttgccaactatgacccgcgtatgaagcgtgaaggcctgcattatgtcgtgattgagcgggatgaaaagtacatggcgagttttgacgagatcgtgccggagttcatcgaaaaaatggacgaggcactggctgaaattggttttgtatttggggagcaatggcgatctggctctggttccggcagcggttccgga

SEQ ID NO: 17 - protein, 226 aa, Artificial Sequence
  bacteriophage lambda exo (redX)
MTPDIILQRTGIDVRAVEQGDDAWHKLRLGVITASEVHNVIAKPRSGKKWPDMKMSYFHTLLAEVCTGVAPEVNAKALAWGKQYENDARTLFEFTSGVNVTESPIIYRDESMRTACSPDGLCSDGNGLELKCPFTSRDFMKFRLGGFEAIKSAYMAQVQYSMWVTRKNAWYFANYDPRMKREGLHYVVIERDEKYMASFDEIVPEFIEKMDEALAEIGFVFGEQWR

SEQ ID NO: 18 - protein, 760 aa, Artificial Sequence
  Hel308 Mbu
MMIRELDIPRDIIGFYEDSGIKELYPPQAEAIEMGLLEKKNLLAAIPTASGKTLLAELAMIKAIREGGKALYIVPLRALASEKFERFKELAPFGIKVGISTGDLDSRADWLGVNDIIVATSEKTDSLLRNGTSWMDEITTVVVDEIHLLDSKNRGPTLEVTITKLMRLNPDVQVVALSATVGNAREMADWLGAALVLSEWRPTDLHEGVLFGDAINFPGSQKKIDRLEKDDAVNLVLDTIKAEGQCLVFESSRRNCAGFAKTASSKVAKILDNDIMIKLAGIAEEVESTGETDTAIVLANCIRKGVAFHHAGLNSNHRKLVENGFRQNLIKVISSTPTLAAGLNLPARRVIIRSYRRFDSNFGMQPIPVLEYKQMAGRAGRPHLDPYGESVLLAKTYDEFAQLMENYVEADAEDIWSKLGTENALRTHVLSTIVNGFASTRQELFDFFGATFFAYQQDKWMLEEVINDCLEFLIDKAMVSETEDIEDASKLFLRGTRLGSLVSMLYIDPLSGSKIVDGFKDIGKSTGGNMGSLEDDKGDDITVTDMTLLHLVCSTPDMRQLYLRNTDYTIVNEYIVAHSDEFHEIPDKLKETDYEWFMGEVKTAMLLEEWVTEVSAEDITRHFNVGEGDIHALADTSEWLMHAAAKLAELLGVEYSSHAYSLEKRIRYGSGLDLMELVGIRGVGRVRARKLYNAGFVSVAKLKGADISVLSKLVGPKVAYNILSGIGVRVNDKHFNSAPISSNTLDTLLDKNQKTFNDFQ

SEQ ID NO: 19 - protein, 707 aa, Artificial Sequence
  Hel308 Csy
MRISELDIPRPAIEFLEGEGYKKLYPPQAAAAKAGLTDGKSVLVSAPTASGKTLIAAIAMISHLSRNRGKAVYLSPLRALAAEKFAEFGKIGGIPLGRPVRVGVSTGDFEKAGRSLGNNDILVLTNERMDSLIRRRPDWMDEVGLVIADEIHLIGDRSRGPTLEMVLTKLRGLRSSPQVVALSATISNADEIAGWLDCTLVHSTWRPVPLSEGVYQDGEVAMGDGSRHEVAATGGGPAVDLAAESVAEGGQSLIFADTRARSASLAAKASAVIPEAKGADAAKLAAAAKKIISSGGETKLAKTLAELVEKGAAFHHAGLNQDCRSVVEEEFRSGRIRLLASTPTLAAGVNLPARRVVISSVMRYNSSSGMSEPISILEYKQLCGRAGRPQYDKSGEAIVVGGVNADEIFDRYIGGEPEPIRSAMVDDRALRIHVLSLVTTSPGIKEDDVTEFFLGTLGGQQSGESTVKFSVAVALRFLQEEGMLGRRGGRLAATKMGRLVSRLYMDPMTAVTLRDAVGEASPGRMHTLGFLHLVSECSEFMPRFALRQKDHEVAEMMLEAGRGELLRPVYSYECGRGLLALHRWIGESPEAKLAEDLKFESGDVHRMVESSGWLLRCIWEISKHQERPDLLGELDVLRSRVAYGIKAELVPLVSIKGIGRVRSRRLFRGGIKGPGDLAAVPVERLSRVEGIGATLANNIKSQLRKGG

SEQ ID NO: 20 - protein, 720 aa, Artificial Sequence
  Hel308 Tga
MKVDELPVDERLKAVLKERGIEELYPPQAEALKSGALEGRNLVLAIPTASGKTLVSEIVMVNKLIQEGGKAVYLVPLKALAEEKYREFKEWEKLGLKVAATTGDYDSTDDWLGRYDIIVATAEKFDSLLRHGARWINDVKLVVADEVHLIGSYDRGATLEMILTHMLGRAQILALSATVGNAEELAEWLDASLVVSDWRPVQLRRGVFHLGTLIWEDGKVESYPENWYSLVVDAVKRGKGALVFVNTRRSAEKEALALSKLVSSHLTKPEKRALESLASQLEDNPTSEKLKRALRGGVAFHHAGLSRVERTLIEDAFREGLIKVITATPTLSAGVNLPSFRVIIRDTKRYAGFGWTDIPVLEIQQMMGRAGRPRYDKYGEAIIVARTDEPGKLMERYIRGKPEKLFSMLANEQAFRSQVLALITNFGIRSFPELVRFLERTFYAHQRKDLSSLEYKAKEVVYFLIENEFIDLDLEDRFIPLPFGKRTSQLYIDPLTAKKFKDAFPAIERNPNPFGIFQLIASTPDMATLTARRREMEDYLDLAYELEDKLYASIPYYEDSRFQGFLGQVKTAKVLLDWINEVPEARIYETYSIDPGDLYRLLELADWLMYSLIELYKLFEPKEEILNYLRDLHLRLRHGVREELLELVRLPNIGRKRARALYNAGFRSVEAIANAKPAELLAVEGIGAKILDGIYRHLGIEKRVTEEKPKRKGTLEDFLR

SEQ ID NO: 21 - protein, 799 aa, Artificial Sequence
  Hel308 Mhu
MEIASLPLPDSFIRACHAKGIRSLYPPQAECIEKGLLEGKNLLISIPTASGKTLLAEMAMWSRIAAGGKCLYIVPLRALASEKYDEFSKKGVIRVGIATGDLDRTDAYLGENDIIVATSEKTDSLLRNRTPWLSQITCIVLDEVHLIGSENRGATLEMVITKLRYTNPVMQIIGLSATIGNPAQLAEWLDATLITSTWRPVDLRQGVYYNGKIRFSDSERPIQGKTKHDDLNLCLDTIEEGGQCLVFVSSRRNAEGFAKKAAGALKAGSPDSKALAQELRRLRDRDEGNVLADCVERGAAFHHAGLIRQERTIIEEGFRNGYIEVIAATPTLAAGLNLPARRVIIRDYNRFASGLGMVPIPVGEYHQMAGRAGRPHLDPYGEAVLLAKDAPSVERLFETFIDAEAERVDSQCVDDASLCAHILSLIATGFAHDQEALSSFMERTFYFFQHPKTRSLPRLVADAIRFLTTAGMVEERENTLSATRLGSLVSRLYLNPCTARLILDSLKSCKTPTLIGLLHVICVSPDMQRLYLKAADTQLLRTFLFKHKDDLILPLPFEQEEEELWLSGLKTALVLTDWADEFSEGMIEERYGIGAGDLYNIVDSGKWLLHGTERLVSVEMPEMSQVVKTLSVRVHHGVKSELLPLVALRNIGRVRARTLYNAGYPDPEAVARAGLSTIARIIGEGIARQVIDEITGVKRSGIHSSDDDYQQKTPELLTDIPGIGKKMAEKLQNAGIITVSDLLTADEVLLSDVLGAARARKVLAFLSNSEKENSSSDKTEEIPDTQKIRGQSSWEDFGC

SEQ ID NO: 22 - protein, 1756 aa, Artificial Sequence
  TraI Eco
MMSIAQVRSAGSAGNYYTDKDNYYVLGSMGERWAGKGAEQLGLQGSVDKDVFTRLLEGRLPDGADLSRMQDGSNKHRPGYDLTFSAPKSVSMMAMLGGDKRLIDAHNQAVDFAVRQVEALASTRVMTDGQSETVLTGNLVMALFNHDTSRDQEPQLHTHAVVANVTQHNGEWKTLSSDKVGKTGFIENVYANQIAFGRLYREKLKEQVEALGYETEVVGKHGMWEMPGVPVEAFSGRSQAIREAVGEDASLKSRDVAALDTRKSKQHVDPEIRMAEWMQTLKETGFDIRAYRDAADQRTEIRTQAPGPASQDGPDVQQAVTQAIAGLSERKVQFTYTDVLARTVGILPPENGVIERARAGIDEAISREQLIPLDREKGLFTSGIHVLDELSVRALSRDIMKQNRVTVHPEKSVPRTAGYSDAVSVLAQDRPSLAIVSGQGGAAGQRERVAELVMMAREQGREVQIIAADRRSQMNLKQDERLSGELITGRRQLLEGMAFTPGSTVIVDQGEKLSLKETLTLLDGAARHNVQVLITDSGQRTGTGSALMAMKDAGVNTYRWQGGEQRPATIISEPDRNVRYARLAGDFAASVKAGEESVAQVSGVREQAILTQAIRSELKTQGVLGHPEVTMTALSPVWLDSRSRYLRDMYRPGMVMEQWNPETRSHDRYVIDRVTAQSHSLTLRDAQGETQVVRISSLDSSWSLFRPEKMPVADGERLRVTGKIPGLRVSGGDRLQVASVSEDAMTVVVPGRAEPASLPVSDSPFTALKLENGWVETPGHSVSDSATVFASVTQMAMDNATLNGLARSGRDVRLYSSLDETRTAEKLARHPSFTVVSEQIKARAGETLLETAISLQKAGLHTPAQQAIHLALPVLESKNLAFSMVDLLTEAKSFAAEGTGFTELGGEINAQIKRGDLLYVDVAKGYGTGLLVSRASYEAEKSILRHILEGKEAVTPLMERVPGELMETLTSGQRAATRMILETSDRFTVVQGYAGVGKTTQFRAVMSAVNMLPASERPRVVGLGPTHRAVGEMRSAGVDAQTLASFLHDTQLQQRSGETPDFSNTLFLLDESSMVGNTEMARAYALIAAGGGRAVASGDTDQLQAIAPGQSFRLQQTRSAADVVIMKEIVRQTPELREAVYSLINRDVERALSGLESVKPSQVPRLEGAWAPEHSVTEFSHSQEAKLAEAQQKAMLKGEAFPDIPMTLYEAIVRDYTGRTPEAREQTLIVTHLNEDRRVLNSMIHDAREKAGELGKEQVMVPVLNTANIRDGELRRLSTWEKNPDALALVDNVYHRIAGISKDDGLITLQDAEGNTRLISPREAVAEGVTLYTPDKIRVGTGDRMRFTKSDRERGYVANSVWTVTAVSGDSVTLSDGQQTRVIRPGQERAEQHIDLAYAITAHGAQGASETFAIALEGTEGNRKLMAGFESAYVALSRMKQHVQVYTDNRQGWTDAINNAVQKGTAHDVLEPKPDREVMNAQRLFSTARELRDVAAGRAVLRQAGLAGGDSPARFIAPGRKYPQPYVALPAFDRNGKSAGIWLNPLTTDDGNGLRGFSGEGRVKGSGDAQFVALQGSRNGESLLADNMQDGVRIARDNPDSGVVVRIAGEGRPWNPGAITGGRVWGDIPDNSVQPGAGNGEPVTAEVLAQRQAEEAIRRETERRADEIVRKMAENKPDLPDGKTELAVRDIAGQERDRSAISERETALPESVLRESQREREAVREVARENLLQERLQQMERDMVRDLQKEKTLGGD

SEQ ID NO: 23 - protein, 726 aa, Artificial Sequence
  XPD Mbu
MSDKPAFMKYFTQSSCYPNQQEAMDRIHSALMQQQLVLFEGACGTGKTLSALVPALHVGKMLGKTVIIATNVHQQMVQFINEARDIKKVQDVKVAVIKGKTAMCPQEADYEECSVKRENTFELMETEREIYLKRQELNSARDSYKKSHDPAFVTLRDELSKEIDAVEEKARGLRDRACNDLYEVLRSDSEKFREWLYKEVRSPEEINDHAIKDGMCGYELVKRELKHADLLICNYHHVLNPDIFSTVLGWIEKEPQETIVIFDEAHNLESAARSHSSLSLTEHSIEKAITELEANLDLLADDNIHNLFNIFLEVISDTYNSRFKFGERERVRKNWYDIRISDPYERNDIVRGKFLRQAKGDFGEKDDIQILLSEASELGAKLDETYRDQYKKGLSSVMKRSHIRYVADFMSAYIELSHNLNYYPILNVRRDMNDEIYGRVELFTCIPKNVTEPLFNSLFSVILMSATLHPFEMVKKTLGITRDTCEMSYGTSFPEEKRLSIAVSIPPLFAKNRDDRHVTELLEQVLLDSIENSKGNVILFFQSAFEAKRYYSKIEPLVNVPVFLDEVGISSQDVREEFFSIGEENGKAVLLSYLWGTLSEGIDYRDGRGRTVIIIGVGYPALNDRMNAVESAYDHVFGYGAGWEFAIQVPTIRKIRQAMGRVVRSPTDYGARILLDGRFLTDSKKRFGKFSVFEVFPPAERSEFVDVDPEKVKYSLMNFFMDNDEQ

SEQ ID NO: 24 - protein, 439 aa, Artificial Sequence
  Dda 1993
MTFDDLTEGQKNAFNIVMKAIKEKKHHVTINGPAGTGKTTLTKFIIEALISTGETGIILAAPTHAAKKILSKLSGKEASTIHSILKINPVTYEENVLFEQKEVPDLAKCRVLICDEVSMYDRKLFKILLSTIPPWCTIIGIGDNKQIRPVDPGENTAYISPFFTHKDFYQCELTEVKRSNAPIIDVATDVRNGKWIYDKVVDGHGVRGFTGDTALRDFMVNYFSIVKSLDDLFENRVMAFTNKSVDKLNSIIRKKIFETDKDFIVGEIIVMQEPLFKTYKIDGKPVSEIIFNNGQLVRIIEAEYTSTFVKARGVPGEYLIRHWDLTVETYGDDEYYREKIKIISSDEELYKFNLFLGKTAETYKNWNKGGKAPWSDFWDAKSQFSKVKALPASTFHKAQGMSVDRAFIYTPCIHYADVELAQQLLYVGVTRGRYDVFYV

SEQ ID NO: 25 - protein, 970 aa, Artificial Sequence
  TrwC Cba
MLSVANVRSPSAAASYFASDNYYASADADRSGQWIGDGAKRLGLEGKVEARAFDALLRGELPDGSSVGNPGQAHRPGTDLTFSVPKSWSLLALVGKDERIIAAYREAVVEALHWAEKNAAETRVVEKGMVVTQATGNLAIGLFQHDTNRNQEPNLHFHAVIANVTQGKDGKWRTLKNDRLWQLNTTLNSIAMARFRVAVEKLGYEPGPVLKHGNFEARGISREQVMAFSTRRKEVLEARRGPGLDAGRIAALDTRASKEGIEDRATLSKQWSEAAQSIGLDLKPLVDRARTKALGQGMEATRIGSLVERGRAWLSRFAAHVRGDPADPLVPPSVLKQDRQTIAAAQAVASAVRHLSQREAAFERTALYKAALDFGLPTTIADVEKRTRALVRSGDLIAGKGEHKGWLASRDAVVTEQRILSEVAAGKGDSSPAITPQKAAASVQAAALTGQGFRLNEGQLAAARLILISKDRTIAVQGIAGAGKSSVLKPVAEVLRDEGHPVIGLAIQNTLVQMLERDTGIGSQTLARFLGGWNKLLDDPGNVALRAEAQASLKDHVLVLDEASMVSNEDKEKLVRLANLAGVHRLVLIGDRKQLGAVDAGKPFALLQRAGIARAEMATNLRARDPVVREAQAAAQAGDVRKALRHLKSHTVEARGDGAQVAAETWLALDKETRARTSIYASGRAIRSAVNAAVQQGLLASREIGPAKMKLEVLDRVNTTREELRHLPAYRAGRVLEVSRKQQALGLFIGEYRVIGQDRKGKLVEVEDKRGKRFRFDPARIRAGKGDDNLTLLEPRKLEIHEGDRIRWTRNDHRRGLFNADQARVVEIANGKVTFETSKGDLVELKKDDPMLKRIDLAYALNVHMAQGLTSDRGIAVMDSRERNLSNQKTFLVTVTRLRDHLTLVVDSADKLGAAVARNKGEKASAIEVTGSVKPTATKGSGVDQPKSVEANKAEKELTRSKSKTLDFGI

SEQ ID NO: 26 - DNA, 786 bp, Artificial Sequence
  WT CsgG from E. coli Str. K-12 substr. MC4100
tgtctgaccgcaccgccgaaagaagcggcacgtccgaccctgatgccgcgtgcacagtcttataaagatctgacccatctgccggctccgacgggcaaaatttttgttagcgtctataacatccaggacgaaaccggtcaatttaaaccgtacccggcgagtaatttctccacggccgttccgcagagtgcaaccgctatgctggtcacggcactgaaagattcccgttggttcattccgctggaacgccagggcctgcaaaacctgctgaatgaacgtaaaattatccgcgcagctcaggaaaacggtaccgtggccattaacaatcgtattccgctgcaaagcctgaccgccgcaaacatcatggttgaaggctctatcatcggttacgaatcaaacgtcaaatcgggcggtgtgggcgcacgttattttggcattggtgctgatacccagtaccaactggaccagatcgcagttaacctgcgcgtggttaatgtcagcaccggcgaaattctgagctctgtgaataccagcaaaacgatcctgtcttacgaagtgcaggctggtgtttttcgtttcattgattatcaacgcctgctggaaggcgaagtcggttacacctcaaacgaaccggtgatgctgtgtctgatgtcggcgattgaaacgggtgttattttcctgatcaatgatggcatcgaccgtggtctgtgggatctgcagaacaaagccgaacgtcaaaatgacattctggtgaaataccgccacatgagtgttccgccggaatcc

SEQ ID NO: 27 - protein, 262 aa, Artificial Sequence
  WT CsgG from E. coli Str. K-12 substr. MC4100
CLTAPPKEAARPTLMPRAQSYKDLTHLPAPTGKIFVSVYNIQDETGQFKPYPASNFSTAVPQSATAMLVTALKDSRWFIPLERQGLQNLLNERKIIRAAQENGTVAINNRIPLQSLTAANIMVEGSIIGYESNVKSGGVGARYFGIGADTQYQLDQIAVNLRVVNVSTGEILSSVNTSKTILSYEVQAGVFRFIDYQRLLEGEVGYTSNEPVMLCLMSAIETGVIFLINDGIDRGLWDLQNKAERQNDILVKYRHMSVPPES

SEQ ID NO: 28 - DNA, 3670 bp, Artificial Sequence
  DNA sequence 1 corrected
  misc_feature (47)..(50): n is iSpC3; C3 phosphoramidite spacer
  misc_feature (78)..(81): n is i5NitInd; 5-Nitroindole, universal base
ttttttttttttttttttttttttttttttttttttttttttttttnnnnggttgtttctgttggtgctgatattgcnnnngccatcagattgtgtttgttagtcgctgccatcagattgtgtttgttagtcgctttttttttttggaattttttttttggaattttttttttgcgctaacaacctcctgccgttttgcccgtgcatatcggtcacgaacaaatctgattactaaacacagtagcctggatttgttctatcagtaatcgaccttattcctaattaaatagagcaaatccccttattgggggtaagacatgaagatgccagaaaaacatgacctgttggccgccattctcgcggcaaaggaacaaggcatcggggcaatccttgcgtttgcaatggcgtaccttcgcggcagatataatggcggtgcgtttacaaaaacagtaatcgacgcaacgatgtgcgccattatcgcctagttcattcgtgaccttctcgacttcgccggactaagtagcaatctcgcttatataacgagcgtgtttatcggctacatcggtactgactcgattggttcgcttatcaaacgcttcgctgctaaaaaagccggagtagaagatggtagaaatcaataatcaacgtaaggcgttcctcgatatgctggcgtggtcggagggaactgataacggacgtcagaaaaccagaaatcatggttatgacgtcattgtaggcggagagctatttactgattactccgatcaccctcgcaaacttgtcacgctaaacccaaaactcaaatcaacaggcgccggacgctaccagcttctttcccgttggtgggatgcctaccgcaagcagcttggcctgaaagacttctctccgaaaagtcaggacgctgtggcattgcagcagattaaggagcgtggcgctttacctatgattgatcgtggtgatatccgtcaggcaatcgaccgttgcagcaatatctgggcttcactgccgggcgctggttatggtcagttcgagcataaggctgacagcctgattgcaaaattcaaagaagcgggcggaacggtcagagagattgatgtatgagcagagtcaccgcgattatctccgctctggttatctgcatcatcgtctgcctgtcatgggctgttaatcattaccgtgataacgccattacctacaaagcccagcgcgacaaaaatgccagagaactgaagctggcgaacgcggcaattactgacatgcagatgcgtcagcgtgatgttgctgcgctcgatgcaaaatacacgaaggagttagctgatgctaaagctgaaaatgatgctctgcgtgatgatgttgccgctggtcgtcgtcggttgcacatcaaagcagtctgtcagtcagtgcgtgaagccaccaccgcctccggcgtggataatgcagcctccccccgactggcagacaccgctgaacgggattatttcaccctcagagagaggctgatcactatgcaaaaacaactggaaggaacccagaagtatattaatgagcagtgcagatagagttgcccatatcgatgggcaactcatgcaattattgtgagcaatacacacgcgcttccagcggagtataaatgcctaaagtaataaaaccgagcaatccatttacgaatgtttgctgggtttctgttttaacaacattttctgcgccgccacaaattttggctgcatcgacagttttcttctgcccaattccagaaacgaagaaatgatgggtgatggtttcctttggtgctactgctgccggtttgttttgaacagtaaacgtctgttgagcacatcctgtaataagcagggccagcgcagtagcgagtagcatttttttcatggtgttattcccgatgctttttgaagttcgcagaatcgtatgtgtagaaaattaaacaaaccctaaacaatgagttgaaatttcatattgttaatatttattaatgtatgtcaggtgcgatgaatcgtcattgtattcccggattaactatgtccacagccctgacggggaacttctctgcgggagtgtccgggaataattaaaacgatgcacacagggtttagcgcgtacacgtattgcattatgccaacgccccggtgctgacacggaagaaaccggacgttatgatttagcgtggaaagatttgtgtagtgttctgaatgctctcagtaaatagtaatgaattatcaaaggtatagtaatatcttttatgttcatggatatttgtaacccatcggaaaactcctgctttagcaagattttccctgtattgctgaaatgtgatttctcttgatttcaacctatcataggacgtttctataagatgcgtgtttcttgagaatttaacatttacaacctttttaagtccttttattaacacggtgttatcgttttctaacacgatgtgaatattatctgtggctagatagtaaatataatgtgagacgttgtgacgttttagttcagaataaaacaattcacagtctaaatcttttcgcacttgatcgaatatttctttaaaaatggcaacctgagccattggtaaaaccttccatgtgatacgagggcgcgtagtttgcattatcgtttttatcgtttcaatctggtctgacctccttgtgttttgttgatgatttatgtcaaatattaggaatgttttcacttaatagtattggttgcgtaacaaagtgcggtcctgctggcattctggagggaaatacaaccgacagatgtatgtaaggccaacgtgctcaaatcttcatacagaaagatttgaagtaatattttaaccgctagatgaagagcaagcgcatggagcgacaaaatgaataaagaacaatctgctgatgatccctccgtggatctgattcgtgtaaaaaatatgcttaatagcaccatttctatgagttaccctgatgttgtaattgcatgtatagaacataaggtgtctctggaagcattcagagcaattgaggcagcgttggtgaagcacgataataatatgaaggattattccctggtggttgactgatcaccataactgctaatcattcaaactatttagtctgtgacagagccaacacgcagtctgtcactgtcaggaaagtggtaaaactgcaactcaattactgcaatgccctcgtaattaagtgaatttacaatatcgtcctgttcggagggaagaacgcgggatgttcattcttcatcacttttaattgatgtatatgctctcttttctgacgttagtctccgacggcaggcttcaatgacccaggctgagaaattcccggaccctttttgctcaagagcgatgttaatttgttcaatcatttggttaggaaagcggatgttgcgggttgttgttctgcgggttctgttcttcgttgacatgaggttgccccgtattcagtgtcgctgatttgtattgtctgaagttgtttttacgttaagttgatgcagatcaattaatacgatacctgcgtcataattgattatttgacgtggtttgatggcctccacgcacgttgtgatatgtagatgataatcattatcactttacgggtcctttccggtgaaaaaaaaggtaccaaaaaaaacatcgtcgtgagtagtgaaccgtaagcac

SEQ ID NO: 29 - DNA, 3589 bp, Artificial Sequence
  DNA sequence 2 corrected
gtgcttacggttcactactcacgacgatgttttttttggtaccttttttttcaccggaaaggacccgtaaagtgataatgattatcatctacatatcacaacgtgcgtggaggccatcaaaccacgtcaaataatcaattatgacgcaggtatcgtattaattgatctgcatcaacttaacgtaaaaacaacttcagacaatacaaatcagcgacactgaatacggggcaacctcatgtcaacgaagaacagaacccgcagaacaacaacccgcaacatccgctttcctaaccaaatgattgaacaaattaacatcgctcttgagcaaaaagggtccgggaatttctcagcctgggtcattgaagcctgccgtcggagactaacgtcagaaaagagagcatatacatcaattaaaagtgatgaagaatgaacatcccgcgttcttccctccgaacaggacgatattgtaaattcacttaattacgagggcattgcagtaattgagttgcagttttaccactttcctgacagtgacagactgcgtgttggctctgtcacagactaaatagtttgaatgattagcagttatggtgatcagtcaaccaccagggaataatccttcatattattatcgtgcttcaccaacgctgcctcaattgctctgaatgcttccagagacaccttatgttctatacatgcaattacaacatcagggtaactcatagaaatggtgctattaagcatattttttacacgaatcagatccacggagggatcatcagcagattgttctttattcattttgtcgctccatgcgcttgctcttcatctagcggttaaaatattacttcaaatctttctgtatgaagatttgagcacgttggccttacatacatctgtcggttgtatttccctccagaatgccagcaggaccgcactttgttacgcaaccaatactattaagtgaaaacattcctaatatttgacataaatcatcaacaaaacacaaggaggtcagaccagattgaaacgataaaaacgataatgcaaactacgcgccctcgtatcacatggaaggttttaccaatggctcaggttgccatttttaaagaaatattcgatcaagtgcgaaaagatttagactgtgaattgttttattctgaactaaaacgtcacaacgtctcacattatatttactatctagccacagataatattcacatcgtgttagaaaacgataacaccgtgttaataaaaggacttaaaaaggttgtaaatgttaaattctcaagaaacacgcatcttatagaaacgtcctatgataggttgaaatcaagagaaatcacatttcagcaatacagggaaaatcttgctaaagcaggagttttccgatgggttacaaatatccatgaacataaaagatattactatacctttgataattcattactatttactgagagcattcagaacactacacaaatctttccacgctaaatcataacgtccggtttcttccgtgtcagcaccggggcgttggcataatgcaatacgtgtacgcgctaaaccctgtgtgcatcgttttaattattcccggacactcccgcagagaagttccccgtcagggctgtggacatagttaatccgggaatacaatgacgattcatcgcacctgacatacattaataaatattaacaatatgaaatttcaactcattgtttagggtttgtttaattttctacacatacgattctgcgaacttcaaaaagcatcgggaataacaccatgaaaaaaatgctactcgctactgcgctggccctgcttattacaggatgtgctcaacagacgtttactgttcaaaacaaaccggcagcagtagcaccaaaggaaaccatcacccatcatttcttcgtttctggaattgggcagaagaaaactgtcgatgcagccaaaatttgtggcggcgcagaaaatgttgttaaaacagaaacccagcaaacattcgtaaatggattgctcggttttattactttaggcatttatactccgctggaagcgcgtgtgtattgctcacaataattgcatgagttgcccatcgatatgggcaactctatctgcactgctcattaatatacttctgggttccttccagttgtttttgcatagtgatcagcctctctctgagggtgaaataatcccgttcagcggtgtctgccagtcggggggaggctgcattatccacgccggaggcggtggtggcttcacgcactgactgacagactgctttgatgtgcaaccgacgacgaccagcggcaacatcatcacgcagagcatcattttcagctttagcatcagctaactccttcgtgtattttgcatcgagcgcagcaacatcacgctgacgcatctgcatgtcagtaattgccgcgttcgccagcttcagttctctggcatttttgtcgcgctgggctttgtaggtaatggcgttatcacggtaatgattaacagcccatgacaggcagacgatgatgcagataaccagagcggagataatcgcggtgactctgctcatacatcaatctctctgaccgttccgcccgcttctttgaattttgcaatcaggctgtcagccttatgctcgaactgaccataaccagcgcccggcagtgaagcccagatattgctgcaacggtcgattgcctgacggatatcaccacgatcaatcataggtaaagcgccacgctccttaatctgctgcaatgccacagcgtcctgacttttcggagagaagtctttcaggccaagctgcttgcggtaggcatcccaccaacgggaaagaagctggtagcgtccggcgcctgttgatttgagttttgggtttagcgtgacaagtttgcgagggtgatcggagtaatcagtaaatagctctccgcctacaatgacgtcataaccatgatttctggttttctgacgtccgttatcagttccctccgaccacgccagcatatcgaggaacgccttacgttgattattgatttctaccatcttctactccggcttttttagcagcgaagcgtttgataagcgaaccaatcgagtcagtaccgatgtagccgataaacacgctcgttatataagcgagattgctacttagtccggcgaagtcgagaaggtcacgaatgaactaggcgataatggcgcacatcgttgcgtcgattactgtttttgtaaacgcaccgccattatatctgccgcgaaggtacgccattgcaaacgcaaggattgccccgatgccttgttcctttgccgcgagaatggcggccaacaggtcatgtttttctggcatcttcatgtcttacccccaataaggggatttgctctatttaattaggaataaggtcgattactgatagaacaaatccaggctactgtgtttagtaatcagatttgttcgtgaccgatatgcacgggcaaaacggcaggaggttgttagcgcaaaaaaaaaattccaaaaaaaaaattccaaaaaaaaaaagcgactaacaaacacaatctgatggcagcgactaacaaacacaatctgatggc

SEQ ID NO: 30 - DNA, 3580 bp, Artificial Sequence
  DNA sequence 1 as in priority document
  misc_feature (47)..(50): n is iSpC3; C3 phosphoramidite spacer
  misc_feature (78)..(81): n is i5NitInd; 5-Nitroindole, universal base
ttttttttttttttttttttttttttttttttttttttttttttttnnnnggttgtttctgttggtgctgatattgcnnnngccatcagattgtgtttgttagtcgctttttttttttggaattttttttttggaattttttttttgcgctaacaacctcctgccgttttgcccgtgcatatcggtcacgaacaaatctgattactaaacacagtagcctggatttgttctatcagtaatcgaccttattcctaattaaatagagcaaatccccttattgggggtaagacatgaagatgccagaaaaacatgacctgttggccgccattctcgcggcaaaggaacaaggcatcggggcaatccttgcgtttgcaatggcgtaccttcgcggcagatataatggcggtgcgtttacaaaaacagtaatcgacgcaacgatgtgcgccattatcgcctagttcattcgtgaccttctcgacttcgccggactaagtagcaatctcgcttatataacgagcgtgtttatcggctacatcggtactgactcgattggttcgcttatcaaacgcttcgctgctaaaaaagccggagtagaagatggtagaaatcaataatcaacgtaaggcgttcctcgatatgctggcgtggtcggagggaactgataacggacgtcagaaaaccagaaatcatggttatgacgtcattgtaggcggagagctatttactgattactccgatcaccctcgcaaacttgtcacgctaaacccaaaactcaaatcaacaggcgccggacgctaccagcttctttcccgttggtgggatgcctaccgcaagcagcttggcctgaaagacttctctccgaaaagtcaggacgctgtggcattgcagcagattaaggagcgtggcgctttacctatgattgatcgtggtgatatccgtcaggcaatcgaccgttgcagcaatatctgggcttcactgccgggcgctggttatggtcagttcgagcataaggctgacagcctgattgcaaaattcaaagaagcgggcggaacggtcagagagattgatgtatgagcagagtcaccgcgattatctccgctctggttatctgcatcatcgtctgcctgtcatgggctgttaatcattaccgtgataacgccattacctacaaagcccagcgcgacaaaaatgccagagaactgaagctggcgaacgcggcaattactgacatgcagatgcgtcagcgtgatgttgctgcgctcgatgcaaaatacacgaaggagttagctgatgctaaagctgaaaatgatgctctgcgtgatgatgttgccgctggtcgtcgtcggttgcacatcaaagcagtctgtcagtcagtgcgtgaagccaccaccgcctccggcgtggataatgcagcctccccccgactggcagacaccgctgaacgggattatttcaccctcagagagaggctgatcactatgcaaaaacaactggaaggaacccagaagtatattaatgagcagtgcagatagagttgcccatatcgatgggcaactcatgcaattattgtgagcaatacacacgcgcttccagcggagtataaatgcctaaagtaataaaaccgagcaatccatttacgaatgtttgctgggtttctgttttaacaacattttctgcgccgccacaaattttggctgcatcgacagttttcttctgcccaattccagaaacgaagaaatgatgggtgatggtttcctttggtgctactgctgccggtttgttttgaacagtaaacgtctgttgagcacatcctgtaataagcagggccagcgcagtagcgagtagcatttttttcatggtgttattcccgatgctttttgaagttcgcagaatcgtatgtgtagaaaattaaacaaaccctaaacaatgagttgaaatttcatattgttaatatttattaatgtatgtcaggtgcgatgaatcgtcattgtattcccggattaactatgtccacagccctgacggggaacttctctgcgggagtgtccgggaataattaaaacgatgcacacagggtttagcgcgtacacgtattgcattatgccaacgccccggtgctgacacggaagaaaccggacgttatgatttagcgtggaaagatttgtgtagtgttctgaatgctctcagtaaatagtaatgaattatcaaaggtatagtaatatcttttatgttcatggatatttgtaacccatcggaaaactcctgctttagcaagattttccctgtattgctgaaatgtgatttctcttgatttcaacctatcataggacgtttctataagatgcgtgtttcttgagaatttaacatttacaacctttttaagtccttttattaacacggtgttatcgttttctaacacgatgtgaatattatctgtggctagatagtaaatataatgtgagacgttgtgacgttttagttcagaataaaacaattcacagtctaaatcttttcgcacttgatcgaatatttctttaaaaatggcaacctgagccattggtaaaaccttccatgtgatacgagggcgcgtagtttgcattatcgtttttatcgtttcaatctggtctgacctccttgtgttttgttgatgatttatgtcaaatattaggaatgttttcacttaatagtattggttgcgtaacaaagtgcggtcctgctggcattctggagggaaatacaaccgacagatgtatgtaaggccaacgtgctcaaatcttcatacagaaagatttgaagtaatattttaaccgctagatgaagagcaagcgcatggagcgacaaaatgaataaagaacaatctgctgatgatccctccgtggatctgattcgtgtaaaaaatatgcttaatagcaccatttctatgagttaccctgatgttgtaattgcatgtatagaacataaggtgtctctggaagcattcagagcaattgaggcagcgttggtgaagcacgataataatatgaaggattattccctggtggttgactgatcaccataactgctaatcattcaaactatttagtctgtgacagagccaacacgcagtctgtcactgtcaggaaagtggtaaaactgcaactcaattactgcaatgccctcgtaattaagtgaatttacaatatcgtcctgttcggagggaagaacgcgggatgttcattcttcatcacttttaattgatgtatatgctctcttttctgacgttagtctccgacggcaggcttcaatgacccaggctgagaaattcccggaccctttttgctcaagagcgatgttaatttgttcaatcatttggttaggaaagcggatgttgcgggttgttgttctgcgggttctgttcttcgttgacatgaggttgccccgtattcagtgtcgctgatttgtattgtctgaagttgtttttacgttaagttgatgcagatcaattaatacgatacctgcgtcataattgattatttgacgtggtttgatggcctccacgcacgttgtgatatgtagatgataatcattatcactttacggg

SEQ ID NO: 31 - DNA, 3525 bp, Artificial Sequence
  DNA sequence 2 as in priority document
ggtaccttttttttcaccggaaaggacccgtaaagtgataatgattatcatctacatatcacaacgtgcgtggaggccatcaaaccacgtcaaataatcaattatgacgcaggtatcgtattaattgatctgcatcaacttaacgtaaaaacaacttcagacaatacaaatcagcgacactgaatacggggcaacctcatgtcaacgaagaacagaacccgcagaacaacaacccgcaacatccgctttcctaaccaaatgattgaacaaattaacatcgctcttgagcaaaaagggtccgggaatttctcagcctgggtcattgaagcctgccgtcggagactaacgtcagaaaagagagcatatacatcaattaaaagtgatgaagaatgaacatcccgcgttcttccctccgaacaggacgatattgtaaattcacttaattacgagggcattgcagtaattgagttgcagttttaccactttcctgacagtgacagactgcgtgttggctctgtcacagactaaatagtttgaatgattagcagttatggtgatcagtcaaccaccagggaataatccttcatattattatcgtgcttcaccaacgctgcctcaattgctctgaatgcttccagagacaccttatgttctatacatgcaattacaacatcagggtaactcatagaaatggtgctattaagcatattttttacacgaatcagatccacggagggatcatcagcagattgttctttattcattttgtcgctccatgcgcttgctcttcatctagcggttaaaatattacttcaaatctttctgtatgaagatttgagcacgttggccttacatacatctgtcggttgtatttccctccagaatgccagcaggaccgcactttgttacgcaaccaatactattaagtgaaaacattcctaatatttgacataaatcatcaacaaaacacaaggaggtcagaccagattgaaacgataaaaacgataatgcaaactacgcgccctcgtatcacatggaaggttttaccaatggctcaggttgccatttttaaagaaatattcgatcaagtgcgaaaagatttagactgtgaattgttttattctgaactaaaacgtcacaacgtctcacattatatttactatctagccacagataatattcacatcgtgttagaaaacgataacaccgtgttaataaaaggacttaaaaaggttgtaaatgttaaattctcaagaaacacgcatcttatagaaacgtcctatgataggttgaaatcaagagaaatcacatttcagcaatacagggaaaatcttgctaaagcaggagttttccgatgggttacaaatatccatgaacataaaagatattactatacctttgataattcattactatttactgagagcattcagaacactacacaaatctttccacgctaaatcataacgtccggtttcttccgtgtcagcaccggggcgttggcataatgcaatacgtgtacgcgctaaaccctgtgtgcatcgttttaattattcccggacactcccgcagagaagttccccgtcagggctgtggacatagttaatccgggaatacaatgacgattcatcgcacctgacatacattaataaatattaacaatatgaaatttcaactcattgtttagggtttgtttaattttctacacatacgattctgcgaacttcaaaaagcatcgggaataacaccatgaaaaaaatgctactcgctactgcgctggccctgcttattacaggatgtgctcaacagacgtttactgttcaaaacaaaccggcagcagtagcaccaaaggaaaccatcacccatcatttcttcgtttctggaattgggcagaagaaaactgtcgatgcagccaaaatttgtggcggcgcagaaaatgttgttaaaacagaaacccagcaaacattcgtaaatggattgctcggttttattactttaggcatttatactccgctggaagcgcgtgtgtattgctcacaataattgcatgagttgcccatcgatatgggcaactctatctgcactgctcattaatatacttctgggttccttccagttgtttttgcatagtgatcagcctctctctgagggtgaaataatcccgttcagcggtgtctgccagtcggggggaggctgcattatccacgccggaggcggtggtggcttcacgcactgactgacagactgctttgatgtgcaaccgacgacgaccagcggcaacatcatcacgcagagcatcattttcagctttagcatcagctaactccttcgtgtattttgcatcgagcgcagcaacatcacgctgacgcatctgcatgtcagtaattgccgcgttcgccagcttcagttctctggcatttttgtcgcgctgggctttgtaggtaatggcgttatcacggtaatgattaacagcccatgacaggcagacgatgatgcagataaccagagcggagataatcgcggtgactctgctcatacatcaatctctctgaccgttccgcccgcttctttgaattttgcaatcaggctgtcagccttatgctcgaactgaccataaccagcgcccggcagtgaagcccagatattgctgcaacggtcgattgcctgacggatatcaccacgatcaatcataggtaaagcgccacgctccttaatctgctgcaatgccacagcgtcctgacttttcggagagaagtctttcaggccaagctgcttgcggtaggcatcccaccaacgggaaagaagctggtagcgtccggcgcctgttgatttgagttttgggtttagcgtgacaagtttgcgagggtgatcggagtaatcagtaaatagctctccgcctacaatgacgtcataaccatgatttctggttttctgacgtccgttatcagttccctccgaccacgccagcatatcgaggaacgccttacgttgattattgatttctaccatcttctactccggcttttttagcagcgaagcgtttgataagcgaaccaatcgagtcagtaccgatgtagccgataaacacgctcgttatataagcgagattgctacttagtccggcgaagtcgagaaggtcacgaatgaactaggcgataatggcgcacatcgttgcgtcgattactgtttttgtaaacgcaccgccattatatctgccgcgaaggtacgccattgcaaacgcaaggattgccccgatgccttgttcctttgccgcgagaatggcggccaacaggtcatgtttttctggcatcttcatgtcttacccccaataaggggatttgctctatttaattaggaataaggtcgattactgatagaacaaatccaggctactgtgtttagtaatcagatttgttcgtgaccgatatgcacgggcaaaacggcaggaggttgttagcgcaaaaaaaaaattccaaaaaaaaaattccaaaaaaaaaaagcgactaacaaacacaatctgatggc

SEQ ID NO: 32 - DNA, 36 bp, Artificial Sequence
  DNA sequence 3
  misc_feature (29)..(34): n is iSp18; 18-atom hexa-ethyleneglycol spacer
  misc_feature (36)..(36): conjugated to 3CholTEG; 3' Cholesteryl-TEG
gcaatatcagcaccaacagaaacaacctnnnnnntt

SEQ ID NO: 33 - DNA, 88 bp, Artificial Sequence
  DNA sequence 4
  misc_feature (50)..(53): n is iSpC3; C3 phosphoramidite spacer
cgttctgtttatgtttcttgtttgttagcctttttttttttttttttttnnnntttttggctaacaaacaagaaacataaacagaacg

SEQ ID NO: 34 - DNA, 10 bp, Artificial Sequence
  AE202
  misc_feature (1)..(1): conjugated to  5CholTEG; 5' Cholesteryl-TEG
  misc_feature (1)..(10): i is inosine
nnnnnnnnnn

SEQ ID NO: 35 - DNA, 115 bp, Artificial Sequence
  AE186
caaataagaacattatgatcagtagggctaacaaacaagaaacataaacagaacgtgcttacggttcactactcacgacgatgttttttttggtaccttttttttcaccggaaag

SEQ ID NO: 36 - DNA, 34 bp, Artificial Sequence
  TE60 corrected
  misc_feature (27)..(32): n is iSp18; 18-atom hexa-ethyleneglycol spacer
  misc_feature (34)..(34): conjugated to 3CholTEG; 3' Cholesteryl-TEG
ctactgatcataatgttcttatttgtnnnnnntt

SEQ ID NO: 37 - DNA, 23 bp, Artificial Sequence
  TE60 as in priority document
  misc_feature (16)..(21): n is iSp18; 18-atom hexa-ethyleneglycol spacer
  misc_feature (23)..(23): conjugated to 3CholTEG; 3' Cholesteryl-TEG
gcaatatcagcacctnnnnnntt

SEQ ID NO: 38 - DNA, 20 bp, Artificial Sequence
  AE203
  misc_feature (1)..(1): conjugated to 5CholTEG; 5' Cholesteryl-TEG
  misc_feature (1)..(20): n is inosine (i)
nnnnnnnnnnnnnnnnnnnn

SEQ ID NO: 39 - DNA, 30 bp, Artificial Sequence
  AE210
  misc_feature (1)..(1): conjugated to 5' Biotin dT
  misc_feature (1)..(30): n is inosine (i)
  misc_feature (30)..(30): conjugated to 5CholTEG; 5' Cholesteryl-TEG
nnnnnnnnnnnnnnnnnnnnnnnnnnnnnn

SEQ ID NO: 40 - DNA, 10 bp, Artificial Sequence
  AE191
  misc_feature (1)..(1): conjugated to 5' Biotin dT
  misc_feature (1)..(10): n is inosine (i)
nnnnnnnnnn

SEQ ID NO: 41 - DNA, 20 bp, Artificial Sequence
  AE192
  misc_feature (1)..(1): is conjugated to 5' Biotin dT
  misc_feature (1)..(20): n is inosine (i)
nnnnnnnnnnnnnnnnnnnn

SEQ ID NO: 42 - DNA, 30 bp, Artificial Sequence; identical to SEQ ID NO: 39
  AE193
  misc_feature (1)..(1): is conjugated to 5' Biotin dT
  misc_feature (1)..(30): n is inosine (i)

SEQ ID NO: 43 - DNA, 40 bp, Artificial Sequence
  AE263
gggtccgggaatttctcagcctgggtcattgaagcctgcc

SEQ ID NO: 44 - DNA, 40 bp, Artificial Sequence
  AE264
ccaaatgattgaacaaattaacatcgctcttgagcaaaaa

SEQ ID NO: 45 - DNA, 40 bp, Artificial Sequence
  AE265
gaacccgcagaacaacaacccgcaacatccgctttcctaa

SEQ ID NO: 46 - DNA, 40 bp, Artificial Sequence
  AE266
cgacactgaatacggggcaacctcatgtcaacgaagaaca

SEQ ID NO: 47 - DNA, 40 bp, Artificial Sequence
  AE267
tcaacttaacgtaaaaacaacttcagacaatacaaatcag

SEQ ID NO: 48 - DNA, 40 bp, Artificial Sequence
  AE268
taatcaattatgacgcaggtatcgtattaattgatctgca

SEQ ID NO: 49 - DNA, 40 bp, Artificial Sequence
  AE269
catatcacaacgtgcgtggaggccatcaaaccacgtcaaa

SEQ ID NO: 50 - DNA, 40 bp, Artificial Sequence
  AE270
caccggaaaggacccgtaaagtgataatgattatcatcta

SEQ ID NO: 51 - DNA, 40 bp, Artificial Sequence
  AE271
tcactactcacgacgatgttttttttggtacctttttttt

SEQ ID NO: 52 - DNA, 40 bp, Artificial Sequence
  AE272
ggctaacaaacaagaaacataaacagaacgtgcttacggt

SEQ ID NO: 53 - DNA, 20 bp, Artificial Sequence
  AE273
ctgggtcattgaagcctgcc

SEQ ID NO: 54 - DNA, 20 bp, Artificial Sequence
  AE274
gggtccgggaatttctcagc

SEQ ID NO: 55 - DNA, 20 bp, Artificial Sequence
  AE275
acatcgctcttgagcaaaaa

SEQ ID NO: 56 - DNA, 20 bp, Artificial Sequence
  AE276
ccaaatgattgaacaaatta

SEQ ID NO: 57 - DNA, 20 bp, Artificial Sequence
  AE277
cgcaacatccgctttcctaa

SEQ ID NO: 58 - DNA, 20 bp, Artificial Sequence
  AE278
gaacccgcagaacaacaacc

SEQ ID NO: 59 - DNA, 20 bp, Artificial Sequence
  AE279
cctcatgtcaacgaagaaca

SEQ ID NO: 60 - DNA, 20 bp, Artificial Sequence
  AE280
cgacactgaatacggggcaa

SEQ ID NO: 61 - DNA, 20 bp, Artificial Sequence
  AE281
cttcagacaatacaaatcag

SEQ ID NO: 62 - DNA, 20 bp, Artificial Sequence
  AE282
tcaacttaacgtaaaaacaa

SEQ ID NO: 63 - DNA, 20 bp, Artificial Sequence
  AE283
atcgtattaattgatctgca

SEQ ID NO: 64 - DNA, 20 bp, Artificial Sequence
  AE284
taatcaattatgacgcaggt

SEQ ID NO: 65 - DNA, 20 bp, Artificial Sequence
  AE285
ggccatcaaaccacgtcaaa

SEQ ID NO: 66 - DNA, 20 bp, Artificial Sequence
  AE286
catatcacaacgtgcgtgga

SEQ ID NO: 67 - DNA, 20 bp, Artificial Sequence
  AE287
gtgataatgattatcatcta

SEQ ID NO: 68 - DNA, 20 bp, Artificial Sequence
  AE288
caccggaaaggacccgtaaa

SEQ ID NO: 69 - DNA, 20 bp, Artificial Sequence
  AE289
ttttttggtacctttttttt

SEQ ID NO: 70 - DNA, 20 bp, Artificial Sequence
  AE290
tcactactcacgacgatgtt

SEQ ID NO: 71 - DNA, 20 bp, Artificial Sequence
  AE291
aaacagaacgtgcttacggt

SEQ ID NO: 72 - DNA, 20 bp, Artificial Sequence
  AE292
ggctaacaaacaagaaacat

SEQ ID NO: 73 - DNA, 80 bp, Artificial Sequence
  AE258
ccaaatgattgaacaaattaacatcgctcttgagcaaaaagggtccgggaatttctcagcctgggtcattgaagcctgcc

SEQ ID NO: 74 - DNA, 80 bp, Artificial Sequence
  AE259
cgacactgaatacggggcaacctcatgtcaacgaagaacagaacccgcagaacaacaacccgcaacatccgctttcctaa

SEQ ID NO: 75 - DNA, 90 bp, Artificial Sequence
  AE182
atctgcactgctcattaatatacttctgggttccttccagttgtttttgcatagtgatcagcctctctctgagggtgaaataatcccgtt

SEQ ID NO: 76 - DNA, 99 bp, Artificial Sequence
  TH14
  misc_feature (1)..(1): is 5' phosphorylated
  misc_feature (49)..(52): n is iSp18; 18-atom hexa-ethyleneglycol spacer
cgtggttggtgtggttggcggacactgattgacacggtttagtagagcnnnntttttttttttttttttttttttcgccaaccacaccaaccacgtcct

SEQ ID NO: 77 - DNA, 99 bp, Artificial Sequence
  TH15
  misc_feature (1)..(1): is 5' phosphorylated
  misc_feature (49)..(52): n is iSp18; 18-atom hexa-ethyleneglycol spacer
cgtccaaccacaccaacccggacactgattgacacggtttagtagagcnnnntttttttttttttttttttttttcgggttggtgtggttggacgtcct

SEQ ID NO: 78 - DNA, 126 bp, Artificial Sequence
  TH16
  misc_feature (1)..(1): is 5' phosphorylated
  misc_feature (62)..(66): n is iSp18; 18-atom hexa-ethyleneglycol spacer
cgtagtccgtggtagggcaggttggggtgaccggacactgattgacacggtttagtagagcnnnntttttttttttttttttttttttcgagtcaccccaacctgccctaccacggactacgtcct

SEQ ID NO: 79 - DNA, 127 bp, Artificial Sequence
  TH17
  misc_feature (1)..(1): is 5' phosphorylated
  misc_feature (63)..(66): n is iSp18; 18-atom hexa-ethyleneglycol spacer
cgtagtcaccccaacctgccctaccacggactcggacactgattgacacggtttagtagagcnnnntttttttttttttttttttttttcgagtccgtggtagggcaggttggggtgactacgtcct

SEQ ID NO: 80 - DNA, 104 bp, Artificial Sequence
  Control hairpin sequence
  misc_feature (1)..(1): is 5' phosphorylated
  misc_feature (49)..(52): n is iSpC3; C3 phosphoramidite spacer
cgtcctgtcgctgtgtctcggacactgattgacacggtttagtagagcnnnnttttttttttttttttttttttttttttcgagacacagcgacaggacgtcct

SEQ ID NO: 81 - DNA, 97 bp, Artificial Sequence
  Y adapter sequence 1
  misc_feature (1)..(30): n is iSpC3; C3 phosphoramidite spacer
  misc_feature (66)..(69): n is iSp18; 18-atom hexa-ethyleneglycol spacer
nnnnnnnnnnnnnnnnnnnnnnnnnnnnnnggcgtctgcttgggtgtttaaccttttttttttttnnnnggttgtttctgttggtgctgatattgct

SEQ ID NO: 82 - DNA, 45 bp, Artificial Sequence
  Y adapter sequence 2
  misc_feature (1)..(1): is 5' phosphorylated
  misc_feature (23)..(23): is iBNA-MeC, where BNA is Bridged Nucleic Acid, where MeC is methyl cytosine
  misc_feature (24)..(24): is iBNA-A, where BNA is Bridged Nucleic Acid
  misc_feature (25)..(25): is iBNA-A, where BNA is Bridged Nucleic Acid
  misc_feature (26)..(26): is iBNA-MeC, where BNA is Bridged Nucleic Acid, where MeC is metylcytosine
  misc_feature (27)..(27): is iBNA-MeC, where BNA is Bridged Nucleic Acid, where MeC is metylcytosine
gcaatatcagcaccaacagaaacaacctttgaggcgagcggtcaa

SEQ ID NO: 83 - DNA, 25 bp, Artificial Sequence
  Y adapter sequence 3
  misc_feature (1)..(1): is iBNA-G, where BNA is Bridged Nucleic Acid
  misc_feature (2)..(2): is iBNA-G, where BNA is Bridged Nucleic Acid
  misc_feature (3)..(3): is iBNA-T, where BNA is Bridged Nucleic Acid
  misc_feature (4)..(4): is iBNA-T, where BNA is Bridged Nucleic Acid
  misc_feature (5)..(5): is iBNA-A, where BNA is Bridged Nucleic Acid
ggttaaacacccaagcagacgcctt